European Patent Specification EP 3 880 843 B1, published September 3, 2025. Title: Method for detection of RNA. Applicant: CartaNA AB. The sequence listing filed with the application follows.

SEQUENCE LISTING (9 sequences)

SEQ ID NO: 1 - DNA, 72 bp, Artificial Sequence
  Hairpin probe
tcattctgcactgatcatctggcatccctgtaagtgtcttctgttattgtgatacagggatgccagatgatc

SEQ ID NO: 2 - DNA, 72 bp, Artificial Sequence
  Hairpin probe
tcattctgcactgatcatctggcatccctgtaagtgtcttctgttattgtgatacatggatgccagatgatc

SEQ ID NO: 3 - DNA, 72 bp, Artificial Sequence
  Hairpin probe
tcattctgcactgatcatctggcatccctgtaagtgtcttctgttattgtgatacattgatgccagatgatc

SEQ ID NO: 4 - DNA, 72 bp, Artificial Sequence
  Hairpin probe
tcattctgcactgatcatctggcatccctgtaagtgtcttctgttattgtgatacagtgatgccatatgatc

SEQ ID NO: 5 - DNA, 73 bp, Artificial Sequence
  Hairpin probe
agcacttgttttgtattgttcaggatttttctgtacaggttctttgggacatcagaaaaatcctgaacaatac

SEQ ID NO: 6 - DNA, 81 bp, Artificial Sequence
  Hairpin probe
aaaatattagcacttgttttgtattgttcaggatttttctgtacaggttctttgggacatcagaaaaatcctgaacaatac

SEQ ID NO: 7 - DNA, 47 bp, Artificial Sequence
  Hairpin probe
gacattgaagtatgctgtgtgctctgttgttgttattgcacacagca

SEQ ID NO: 8 - DNA, 55 bp, Artificial Sequence
  Hairpin probe
ctgaaatagacattgaagtatgctgtgtgctctgttgttgttattgcacacagca

SEQ ID NO: 9 - DNA, 60 bp, Artificial Sequence
  Hairpin probe
attctcatagcctggttcctgaacaatacaaaacaagtgcttctaccaggctatgagaat